European Patent Specification EP 4 051 307 B1, published February 1, 2023. Title: TIP-Corona. Applicant: APEPTICO FORSCHUNG UND ENTWICKLUNG GMBH. The sequence listing filed with the application follows.

SEQUENCE LISTING (6 sequences)

SEQ ID NO: 1 - protein, 17 aa, Artificial Sequence
  AP301 peptide
CGQRETPEGAEAKPWYC

SEQ ID NO: 2 - protein, 6 aa, Artificial Sequence
  peptide sequence
TPEGAE

SEQ ID NO: 3 - protein, 14 aa, Artificial Sequence
  peptide
QRETPEGAEAKPWY

SEQ ID NO: 4 - protein, 14 aa, Artificial Sequence
  peptide
PKDTPEGAELKPWY

SEQ ID NO: 5 - protein, 17 aa, Artificial Sequence
  peptide
CGPKDTPEGAELKPWYC

SEQ ID NO: 6 - protein, 6 aa, Artificial Sequence
  peptide sequence
  VARIANT 2,4,5: any natural or non-natural amino-acid
TXEXXE